European Patent Application EP 4 700 130 A1, published February 25, 2026. Title: METHOD FOR PREPARING α-AMINO ACID ESTER ACYLTRANSFERASE AND USE THEREOF IN DIPEPTIDE SYNTHESIS. Applicant: ASYMECHEM LIFE SCIENCE(TIANJIN)CO., LTD. The sequence listing filed with the application follows.

SEQUENCE LISTING (11 sequences)

SEQ ID NO: 1 - protein, 11 aa, Sphingobacterium sp.
YGISYPGFYST

SEQ ID NO: 2 - protein, 619 aa, Sphingobacterium sp.
MKKGITIFSALLIAFSFKAAAQSTAESNYVKEHYEKTEIAIPMRDGVKLFTTIYSPKDKSQSYPVLLNRTPYTVGPYGPNEYKPSLGNFPAMAKEGYIFVYQDVRGKWMSEGTFEDVRPTTLKKGKKDIDESTDTYDLLEWLSKNLKNYNGKAGMYGISYPGFYSTVSLVKTHPSLKAVSPQAPVTNWYIGDDFHHNGVLFTGDAFKFMSSFGIPRPQPITPNQAPHTFQYPSKDVYQFYLTGGTAKDLKNTYFADSVKFWNDAFAHPHYDQFWKDRLILPHLTNVKPAVMIVGGFFDAEDAYGTFETYKKIEEQNPQNKSILVAGPWFHGGWVRSDGSSFGDIQFDQKTSVTYQEKFELPFFNYYLKGKGDFKAAEANIFVTGSNQWKSFDKWPPKDVEDKKLYLQPQGKLDFEKVGRTDSWDEYVSDPNKPVPYQGGVMESRTREYMIDDQRFASSRPDVMVYQTEPLTADITIVGPIKNFLKVSTSGTDADYVVKLIDVYPANSPSFNNKVMDGYQMLVRGEIMAGKYRNSFEKAEPMQPGFVTDIKYTMPDVAHTFKKGHRIMIQVQNTWFPIAERNPQQFFEGYEATATDYRKATHRIFHDVNNASYIEFSVLK

SEQ ID NO: 3 - protein, 619 aa, Sphingobacterium sp.
MKNTISYLTLALLSASQLHAQTAADSAYVRDHYEKTEVAIPMRDGKKLFTAIYSPKDKSKKYPVLLNRTPYTVSPYGQNEYKKSLGNFPQMMHEGYIFVYQDVRGKWMSEGDFEDIRPTTYSKDKKAIDESTDTYDALEWLQKNLKNYNGKAGLYGISYPGFYSTVGLVKTHPSLKAVSPQAPVTDWYIGDDFHHNGVLFLQDAFTFMSTFGVPRPKPITPDQFKGKIQIKEADKYNFFAEAGTARELKEKYFGDSVQFWNDLFKHPDYDDFWKSRVITNSLQEVRPAVMVVGGFFDAEDAYGTFKTYQSIEDKSKKNNSILVAGPWYHGGWVRAEGNYLGDIQFEKKTSITYQEQFEQPFFKYYLKDEGNFAPSEANIFVSGSNEWKHFEQWPPKNVETKKLYFQPQGKLGFDKVQRTDSWDEYVTDPNKPVPHQGGLIQNRTREYMVDDQRFAASRPDVMVYQTEPLTEDLTIVGPIKNFLKVSSTGTDADYVVKLIDVYPNDAASYQGKTMAGYQMMVRGEIMAGKYRNGFDKAQALTPGMVEKVNFEMPDVAHTFKKGHRIMVQVQNSWFPLAERNPQVFLAPYTATKADFRKATQRIFHDVNNATYIEFSVLKD

SEQ ID NO: 4 - protein, 619 aa, Sphingobacterium siyangense
MKNTISCLTLALLSASQLHAQTAADSAYVRDHYEKTEVAIPMRDGKKLFTAIYSPKDKSKKYPVLLNRTPYTVSPYGQNEYKKSLGNFPQMMREGYIFVYQDVRGKWMSEGDFEDIRPTTYNKDKKAIDESTDTYDALEWLQKNLKNYNGKAGLYGISYPGFYSTVGLVKTHPSLKAVSPQAPVTDWYIGDDFHHNGVLFLQDAFTFMSTFGVPRPKPITPDQFKGKIQIKEADKYNFFAEAGTARELKEKYFGDSVQFWNDLFKHPDYDDFWKSRVITNSLQEVKPAVMVVGGFFDAEDAYGTFKTYQSIEDKSKRNNSILVAGPWYHGGWVRAEGNYLGDIQFEKKTSITYQEQFEQPFFKYYLKDEGNFAPAEANIFVSGSNEWKHFEQWPPKNVETKKLYFQPQGKLGFDKVQRTDSWDEYVTDPNKPVPHQGGLIQNRTREYMVDDQRFAASRPDVMVYQTEPLTEDLTIVGPIKNFLKVSSTGTDADYVVKLIDVYPNDAASYQGKTMAGYQMMVRGEIMAGKYRNGFDKAQALTPGMVEKVNFEMPDVAHTFKKGHRIMVQVQNSWFPLAERNPQVFLPSYTATKADFRKATQRIFHDVNNATYIEFSVLKD

SEQ ID NO: 5 - protein, 619 aa, Sphingobacterium sp.
MKNTISYLTLALLSASQLHAQTPADSAYVRDHYEKTEVAIPMRDGKKLFTAIYSPKDKSKKYPVLLNRTPYTVSPYGQNEYKKSLGNFPAMMREGYIFVYQDVRGKWMSEGNFEDIRPTTYSKDKKAFDESTDTYDALEWLQKNLKNYNGKAGLYGISYPGFYSTVGLVKTHPSLKAVSPQAPVTDWYIGDDFHHNGVLFLQDAFTFMSTFGVPRPKPITPDQFKSKIQIKEADKYNFFLEAGTARELKEKYFGDSVQFWNDLFKHPDYDDFWKSRVITNSLQEVKPAVMVVGGFFDAEDAYGTFKTYQSIEDKSKKNNSILVAGPWYHGGWVRAEGNYLGDIQFEKKTSVTYQEQFEQPFFKYYLKDEGNFAPSEANIFVSGSNEWKHFEQWPPKNVEIKKLYFQPQGKLGFDKVQRTDSWDEYVTDPNKPVPHQGGLIQNRTREYMVDDQRFAASRPDVMVYQTEPLTEDLTIVGPIKNFLKVSSTGTDADYVVKLIDVYPNDAASYQGKTMAGYQMMVRGEIMAGKYRNGFEKAQALTPGMVEKVNFEMPDVAHTFKKGHRIMVQVQNSWFPLAERNPQVFLAPYTATKADFRKATQRIFHDVNNATYIEFSVLKD

SEQ ID NO: 6 - protein, 623 aa, Pedobacter sp.
MPRIKHLLFILLFSYGLSASAQNIDSIYVRENYTKIERSIPMRDGVKLFTAIYIPKDQNRKYPFLINRTPYTVAPYGADKYKLSLGNFPAMMREGFIFVYQDVRGKWMSEGTFDDIRPHIANKKSKKQIDESSDTYDTIDWLVKNIKNNNGKAGIYGISYPGFYSTASLPESHPALKAVSPQAPVTDWFIGDDFHHNGVLFLMDAFSFMTTFGVPRPKPITPDLGPKGLKFPIQDNYRFYLEAGSIKNLKDKYMGDSIRFWNNLFAHPNLDTFWQARNIQRHLKSVKPAVMVVGGFFDAEDAYGTFSTYKSIEKQNPSANNILVMGPWYHGGWVRSTGSSFGDIEFGQPTSLQYQERFELPFFKYYLKGQGDFKPAEANIFVTGSNEWKSFGTWPPKDTEQKTLYLQPNGKLSFDKVQRTDSWDEYVSDPNTPVPYQEGVQAKRTREYMIDDQRFAARRPDVKVYQTDALTEDITLTGPVLANLVVSTTGTDADYVVKLIDVYPEDAPAPVPNPKNILMGGFQMLVRGEIMRGKYRNSFEKPEAMVPGLVTKVNYALPDVAHTFRKGHKIMIQVQNSWFPLGDRNPQKFMDIYTAEPSDFQKATQRIFHDVNNASSITISVLK

SEQ ID NO: 7 - protein, 623 aa, Pedobacter sp.
MNLTRIFSLLFCLLIANQLMAQQTDSAYVRENYTKIERQIPMRDGVKLFTSIYIPKNQSKKYPFLINRTPYTVAPYGEDKYKLSLGNFPAMMREGFIFVYQDVRGRWMSEGTFADIRPQQTGKKSKNAIDESTDTYDTIDWLVKNVKGNNGNAGIYGISYPGFYSTTSLPNAHPALKAVSPQAPVTDWFMGDDFHHRGTLFLMDAFSFMGSFGVPRPKPITPDKGPKGFQFPIEDNYRFYLEAGSVKSLKDKYFADSIKFWNDLFKHPNLDTFWKARLITPHLTNVKPAVMVVGGFFDAEDAYGTFATYKAIEKQNPGANNILVAGPWFHGGWVRSDGSSFGDIPFGKTTSIDYQEQYELPFFKHYLKGEGDFNAAEANIFVTGSNEWKKFKTWPPQGVESKNLYLQPNGKLAFEKVGRTDSWDEYVSDPNNPVPYQDGIQSKRTREYMIDDQRFAARRPDVKSYQTDALTEDITLTGPVLANLVVSTTGTDADYVVKLIDVYPEDAPNPEPNPKNLIMGGYEMLVRGEIMRGKYRNSFEKPEAFIPGTITKVNYPLPDVAHTFKKGHKIMIQIQNSWFPLADRNPQKFMDIYQAEPQDFQKATHKIYHDVHNSSYITVSVLK

SEQ ID NO: 8 - protein, 619 aa, Sphingobacterium sp.
MKKVLIIFSVFLITISLQVKAQVTLEPNYVKEHYEKKEIAIPMRDGVKLFTTIYTPKDKSQQYPVLLNRTPYTVGPYGEDKFKESLGNFPAMTTEGYIFVYQDVRGKWMSEGTFEDIRPTNLKKGKREIDESTDTYDLLEWLSKNLQNYNGKAGMYGISYPGFYSTVSLVKTHPSLKAVSPQAPVTNWYMGDDFHHNGILFTGDAFKFMSSFGIPRPKPITPDQAPQTFQYPSKDVYQFYLDAGTAKDLKDKYFADSVKFWNDVFAHPHYDQFWKDREILPHVKNVKPAVMIVGGFFDAEDTYGTFETYKTIEKQNPNNNSILVVGPWFHGGWVRGDGSSFGDIQFDQKTSVTYQEQFELPFFNYYLKGKGDFKASEANIFITGSNQWKAFEKWPPQEVEDKKLYLQPQGKLGFDQVKRTDSWDEYVSDPNKPVPYQAGIMESRTREYMIDDQRFASSRPDVMVYQTEPLAADLTIVGPIKNFLKVSTSGTDADYVVKLIDVYPANSPSFNNKVMDGYQMLVRGEIMAGKYRNGFEKAEAMQPGFVTAIDYTMPDVAHTFKKGHRIMLQVQNTWFPLAERNPQQFFEGYEATAGDYRKATHRIFHDVNNSSYIQFAILK

SEQ ID NO: 9 - protein, 622 aa, Pedobacter sp.
MNLSKILGIVICLFVSHEMFAQQPDSAYVRENYTKIERQIPMRDGVKLFTSIYIPKNQSKKYPFLINRTPYTVAPYGEDKYKLSLGNFPAMMREGFIFVYQDVRGRWMSEGTFEDIRPQTLKKGKKDIDESTDTYDTIDWLVKNIKNNNGNAGIYGISYPGFYSTTSLPNAHPALKAVSPQAPVTDWFIGDDFHHGGALFLMDAFSFMSGFGVPRPKPITPDKGPKGFNFPIQDNYRFYLESGSVKNLKDKYFADSIKFWNNLVKHPNLDTFWKARYIIPHLKNVKPAVMVVGGFFDAEDAYGTFATYKAIEKQNPEANNILVAGPWFHGGWVRSDGASFGDIKFGKTTSIDYQQQFELPFFKHYLKGEGDFKAAEANIFVTGSNEWKKFGSWPPKEVETKNLYLQPNGKLAFEKVGRTDSWDEYVSDPNHPVPYQDGVQAKRTREYMIDDQRFAARRPDVKTYQTDALKDDITLTGPVLANLVVSTTGTDADYVVKLIDVYPEDEPNPSPNPNNIMMGGYEMLVRGEILRGKYRNTFEKPEAFVPGAITKVNYALPDVAHTFKKGHKIMIQIQNSWFPLADRNPQKFMDIYQAEPGDFQKATHKIYHDTSNSSYISVSVLK

SEQ ID NO: 10 - protein, 619 aa, Sphingobacterium multivorum
MKNTISCLTLALLSASQLHAQTAADSAYVRDHYEKTEVAIPMRDGKKLFTAIYSPKDKSKKYPVLLNRTPYTVSPYGQNEYKKSLGNFPQMMREGYIFVYQDVRGKWMSEGDFEDIRPTTYSKDKKAIDESTDTYDALEWLLKNLKNYNGKAGLYGISYPGFYSTVGLVKTHPSLKAVSPQAPVTDWFIGDDFHHNGVLFLQDAFTFMSTFGVPRPKPITPDQFKGKIQIKEADKYNFFAEAGTARELKEKYFGDSVQFWNDLFKHPDYDDFWKSRVITNSLQEVKPAVMVVGGFFDAEDAYGTFKTYQSIEDKSKKNNSILVAGPWYHGGWVRAEGNYLGDIQFEKKTSITYQEQFEQPFFKYYLKDEGNFAPSEANIFVSGSNEWKHFEQWPPKNVETKKLYFQPQGKLGFDKVQRTDSWDEYVTDPNKPVPHQGGLIQNRTREYMVDDQRFAASRPDVMVYQTEPLTEDLTIVGPIKNFLKVSSTGTDADYVVKLIDVYPNDAASYQGKTMAGYQMMVRGEIMAGKYRNGFDKAQALTPGMVEKVNFEMPDVAHTFKKGHRIMVQIQNSWFPLAERNPQVFLAPYTATKADFRKATQRIFHDVNNATYIEFSVLKD

SEQ ID NO: 11 - protein, 619 aa, Sphingobacterium sp.
MKTTISFLALTLFAGGQLHAQTNTDSAYVRDHYEKTEVTVPMRDGKKLFTVIYSPKDKSKKYPILLNRTPYTVGPYGQNEYKKSLGNFPAMMRDGYIFVYQDVRGKWMSEGDFEDVRPTNLSKDKKAIDESTDTYDVLEWLQKNLQNYNGKAGLYGISYPGFYSTVGLVKTHPSLKAVSPQAPVTDWFIGDDFHHNGVLFLQDAFTFMSTFGVPRPKPIRPNQFTSKIQINEVDKYNFFLEAGTARELKEKYFGDSVQFWNNLFKHPNYDDFWKSRVITNYLQDVKPAVMVVGGFFDAEDAYGTFKTYQSIEEKSKTNNSVLVAGPWYHGGWVRAAGDYLGDIQFEKKTSITYQEKFEQPFFSHYLKEEGSFSPAEANIFISGSNEWKQFEQWPPKNVETKKLYFQPQGKLGFEKVQRTDSWDEYVTDPNKPVPHQGGLIQNRTREYMVDDQRFAASRPDVMVYETAPLTEDITIVGPIKNFLKVASTGTDADYIVKLIDVYPSDAPSFDGKPMAGYQMMVRGEIMAGKYRNGFDKPQPLTPGKVEKVDFVMPDVAHTFKKGHRIMVQVQNSWFPLAERNPQVFMAPYTATKTDFRKATQRIFHDVNNATYIEFDILKD